European Patent Application EP 4 696 704 A1, published February 18, 2026. Title: 突变型VSVG及靶向载体. Applicant: 深圳市济因生物科技有限公司. Application WO. The sequence listing filed with the application follows.

SEQUENCE LISTING (30 sequences)

SEQ ID NO: 1 - protein, 495 aa, Vesicular Stomatitis Virus-Indiana
KFTIVFPHNQKGNWKNVPSNYHYCPSSSDLNWHNDLIGTALQVKMPKSHKAIQADGWMCHASKWVTTCDFRWYGPKYITHSIRSFTPSVEQCKESIEQTKQGTWLNPGFPPQSCGYATVTDAEAVIVQVTPHHVLVDEYTGEWVDSQFINGKCSNYICPTVHNSTTWHSDYKVKGLCDSNLISMDITFFSEDGELSSLGKEGTGFRSNYFAYETGGKACKMQYCKHWGVRLPSGVWFEMADKDLFAAARFPECPEGSSISAPSQTSVDVSLIQDVERILDYSLCQETWSKIRAGLPISPVDLSYLAPKNPGTGPAFTIINGTLKYFETRYIRVDIAAPILSRMVGMISGTTTERELWDDWAPYEDVEIGPNGVLRTSSGYKFPLYMIGHGMLDSDLHLSSKAQVFEHPHIQDAASQLPDDESLFFGDTGLSKNPIELVEGWFSSWKSSIASFFFIIGLIIGLFLVLRVGIHLCIKLKHTKKRQIYTDIEMNRLGK

SEQ ID NO: 2 - protein, 495 aa, synthetic construct
KFTIVFPHNQKGNWKNVPSNYHYCPSSSDLNWHNDLIGTALQVKMPKSHKAIQADGWMCHASKWVTTCDFRWYGPKYITHSIRSFTPSVEQCKESIEQTKQGTWLNPGFPPQSCGYATVTDAEAVIVQVTPHHVLVDEYTGEWVDSQFINGKCSNYICPTVHNSTTWHSDYKVKGLCDSNLISMDITFFSEDGELSSLGKEGTGFRSNYFAYENGGKACKMQYCKHWGVRLPSGVWFEMADKDLFAAARFPECPEGSSISAPSQTSVDVSLIQDVERILDYSLCQETWSKIRAGLPISPVDLSYLAPKNPGTGPAFTIINGTLKYFETRYIRVDIAAPILSRMVGMISGTTAEQELWDDWAPYEDVEIGPNGVLRTSSGYKFPLYMIGHGMLDSDLHLSSKAQVFEHPHIQDAASQLPDDESLFFGDTGLSKNPIELVEGWFSSWKSSIASFFFIIGLIIGLFLVLRVGIHLCIKLKHTKKRQIYTDIEMNRLGK

SEQ ID NO: 3 - protein, 495 aa, synthetic construct
KFTIVFPHNQKGNWKNVPSNYHYCPSSSDLNWHNDLIGTALQVKMPKSHTAIQADGWMCHASKWVTTCDFRWYGPKYITHSIRSFTPSVEQCKESIEQTKQGTWLNPGFPPQSCGYATVTDAEAVIVQVTPHHVLVDEYTGEWVDTQFINGKCSNYICPTVHNSTTWHSDYKVKGLCDSNLISMDITFFSEDGELSSLGKEGTGFRSNYFAYENGGKACKMQYCKHWGVRLPSGVWFEMADKDLFAAARFPECPEGSSISAPSQTSVDVSLIQDVERILDYSLCQETWSKIRAGLPISPVDLSYLAPKNPGTGPAFTIINGTLKYFETRYIRVDIAAPILSRMVGMISGTTAEQELWDDWAPYEDVEIGPNGVLRTSSGYKFPLYMIGHGMLDSDLHLSSKAQVFEHPHIQDAASQLPDDESLFFGDTGLSKNPIELVEGWFSSWKSSIASFFFIIGLIIGLFLVLRVGIHLCIKLKHTKKRQIYTDIEMNRLGK

SEQ ID NO: 4 - protein, 21 aa, Homo sapiens
MALPVTALLLPLALLLHAARP

SEQ ID NO: 5 - protein, 117 aa, synthetic construct
EVQLVESGGGLVKPGGSLKLSCAASGLTFSSYAMSWVRQTPEKRLEWVASISSGGFTYYPDSVKGRFTISRDNARNILYLQMSSLRSEDTAMYYCARDEVRGYLDVWGAGTTVTVSS

SEQ ID NO: 6 - protein, 15 aa, synthetic construct
GGGGSGGGGSGGGGS

SEQ ID NO: 7 - protein, 112 aa, synthetic construct
AAYKDIQMTQTTSSLSASLGDRVTISCSASQGISNYLNWYQQKPDGTVKLLIYYTSSLHSGVPSRFSGSGSGTDYSLTISNLEPEDIATYYCQQYSKLPYTFGGGTKLEIKR

SEQ ID NO: 8 - protein, 45 aa, Homo sapiens
TTTPAPRPPTPAPTIASQPLSLRPEACRPAAGGAVHTRGLDFACD

SEQ ID NO: 9 - protein, 24 aa, Homo sapiens
IYIWAPLAGTCGVLLLSLVITLYC

SEQ ID NO: 10 - protein, 495 aa, Vesicular Stomatitis Virus-Cocal
KFSIVFPQSQKGNWKNVPSSYHYCPSSSDQNWHNDLLGITMKVKMPKTHKAIQADGWMCHAAKWITTCDFRWYGPKYITHSIHSIQPTSEQCKESIKQTKQGTWMSPGFPPQNCGYATVTDSVAVVVQATPHHVLVDEYTGEWIDSQFPNGKCETEECETVHNSTVWYSDYKVTGLCDATLVDTEITFFSEDGKKESIGKPNTGYRSNYFAYEKGDKVCKMNYCKHAGVRLPSGVWFEFVDQDVYAAAKLPECPVGATISAPTQTSVDVSLILDVERILDYSLCQETWSKIRSKQPVSPVDLSYLAPKNPGTGPAFTIINGTLKYFETRYIRIDIDNPIISKMVGKISGSQTERELWTEWFPYEGVEIGPNGILKTPTGYKFPLFMIGHGMLDSDLHKTSQAEVFEHPHLAEAPKQLPEEETLFFGDTGISKNPVELIEGWFSSWKSTVVTFFFAIGVFILLYVVARIVIAVRYRYQGSNNKRIYNDIEMSRFRK

SEQ ID NO: 11 - protein, 494 aa, synthetic construct
KFTIVFPHNQKGNWKNVPSNYHYCPSSSDLNWHNDLIGTALQVKMPSHKAIQADGWMCHASKWVTTCDFRWYGPKYITHSIRSFTPSVEQCKESIEQTKQGTWLNPGFPPQSCGYATVTDAEAVIVQVTPHHVLVDEYTGEWVDSQFINGKCSNYICPTVHNSTTWHSDYKVKGLCDSNLISMDITFFSEDGELSSLGKEGTGFRSNYFAYENGGKACKMQYCKHWGVRLPSGVWFEMADKDLFAAARFPECPEGSSISAPSQTSVDVSLIQDVERILDYSLCQETWSKIRAGLPISPVDLSYLAPKNPGTGPAFTIINGTLKYFETRYIRVDIAAPILSRMVGMISGTTAERELWDDWAPYEDVEIGPNGVLRTSSGYKFPLYMIGHGMLDSDLHLSSKAQVFEHPHIQDAASQLPDDESLFFGDTGLSKNPIELVEGWFSSWKSSIASFFFIIGLIIGLFLVLRVGIHLCIKLKHTKKRQIYTDIEMNRLGK

SEQ ID NO: 12 - protein, 494 aa, synthetic construct
KFTIVFPHNQKGNWKNVPSNYHYCPSSSDLNWHNDLIGTALQVKMPSHTAIQADGWMCHASKWVTTCDFRWYGPKYITHSIRSFTPSVEQCKESIEQTKQGTWLNPGFPPQSCGYATVTDAEAVIVQVTPHHVLVDEYTGEWVDTQFINGKCSNYICPTVHNSTTWHSDYKVKGLCDSNLISMDITFFSEDGELSSLGKEGTGFRSNYFAYENGGKACKMQYCKHWGVRLPSGVWFEMADKDLFAAARFPECPEGSSISAPSQTSVDVSLIQDVERILDYSLCQETWSKIRAGLPISPVDLSYLAPKNPGTGPAFTIINGTLKYFETRYIRVDIAAPILSRMVGMISGTTAERELWDDWAPYEDVEIGPNGVLRTSSGYKFPLYMIGHGMLDSDLHLSSKAQVFEHPHIQDAASQLPDDESLFFGDTGLSKNPIELVEGWFSSWKSSIASFFFIIGLIIGLFLVLRVGIHLCIKLKHTKKRQIYTDIEMNRLGK

SEQ ID NO: 13 - protein, 494 aa, synthetic construct
KFSIVFPQSQKGNWKNVPSSYHYCPSSSDQNWHNDLLGITMKVKMPKTHKAIQADGWMCHAAKWITTCDFRWYGPKYITHSIHSIQPTSEQCKESIKQTKQGTWMSPGFPPQNCGYATVTDSVAVVVQATPHHVLVDEYTGEWIDSQFPNGKCETEECETVHNSTVWYSDYKVTGLCDATLVDTEITFFSEDGKKESIGKPNTGYRSNYFAYENGDKVCKMNYCKHAGVRLPSGVWFEFVDQDVYAAAKLPECPVGATISAPTQTSVDVSLILDVERILDYSLCQETWSKIRSKQPVSPVDLSYLAPKNPGTGPAFTIINGTLKYFETRYIRIDIDNPIISKMVGKISGSQAEELWTEWFPYEGVEIGPNGILKTPTGYKFPLFMIGHGMLDSDLHKTSQAEVFEHPHLAEAPKQLPEEETLFFGDTGISKNPVELIEGWFSSWKSTVVTFFFAIGVFILLYVVARIVIAVRYRYQGSNNKRIYNDIEMSRFRK

SEQ ID NO: 14 - protein, 494 aa, synthetic construct
KFSIVFPQSQKGNWKNVPSSYHYCPSSSDQNWHNDLLGITMKVKMPKTHTAIQADGWMCHAAKWITTCDFRWYGPKYITHSIHSIQPTSEQCKESIKQTKQGTWMSPGFPPQNCGYATVTDSVAVVVQATPHHVLVDEYTGEWIDTQFPNGKCETEECETVHNSTVWYSDYKVTGLCDATLVDTEITFFSEDGKKESIGKPNTGYRSNYFAYENGDKVCKMNYCKHAGVRLPSGVWFEFVDQDVYAAAKLPECPVGATISAPTQTSVDVSLILDVERILDYSLCQETWSKIRSKQPVSPVDLSYLAPKNPGTGPAFTIINGTLKYFETRYIRIDIDNPIISKMVGKISGSQAEELWTEWFPYEGVEIGPNGILKTPTGYKFPLFMIGHGMLDSDLHKTSQAEVFEHPHLAEAPKQLPEEETLFFGDTGISKNPVELIEGWFSSWKSTVVTFFFAIGVFILLYVVARIVIAVRYRYQGSNNKRIYNDIEMSRFRK

SEQ ID NO: 15 - protein, 494 aa, synthetic construct
KFTIVFPHNQKGNWKNVPSNYHYCPSSSDLNWHNDLIGTALQVKMPKSHKAIQADGWMCHASKWVTTCDFRWYGPKYITHSIRSFTPSVEQCKESIEQTKQGTWLNPGFPPQSCGYATVTDAEAVIVQVTPHHVLVDEYTGEWVDSQFINGKCSNYICPTVHNSTTWHSDYKVKGLCDSNLISMDITFFSEDGELSSLGKEGTGFRSNYFAYENGGKACKMQYCKHWGVRLPSGVWFEMADKDLFAAARFPECPEGSSISAPSQTSVDVSLIQDVERILDYSLCQETWSKIRAGLPISPVDLSYLAPKNPGTGPAFTIINGTLKYFETRYIRVDIAAPILSRMVGMISGTTAEELWDDWAPYEDVEIGPNGVLRTSSGYKFPLYMIGHGMLDSDLHLSSKAQVFEHPHIQDAASQLPDDESLFFGDTGLSKNPIELVEGWFSSWKSSIASFFFIIGLIIGLFLVLRVGIHLCIKLKHTKKRQIYTDIEMNRLGK

SEQ ID NO: 16 - protein, 494 aa, synthetic construct
KFTIVFPHNQKGNWKNVPSNYHYCPSSSDLNWHNDLIGTALQVKMPKSHTAIQADGWMCHASKWVTTCDFRWYGPKYITHSIRSFTPSVEQCKESIEQTKQGTWLNPGFPPQSCGYATVTDAEAVIVQVTPHHVLVDEYTGEWVDTQFINGKCSNYICPTVHNSTTWHSDYKVKGLCDSNLISMDITFFSEDGELSSLGKEGTGFRSNYFAYENGGKACKMQYCKHWGVRLPSGVWFEMADKDLFAAARFPECPEGSSISAPSQTSVDVSLIQDVERILDYSLCQETWSKIRAGLPISPVDLSYLAPKNPGTGPAFTIINGTLKYFETRYIRVDIAAPILSRMVGMISGTTAEELWDDWAPYEDVEIGPNGVLRTSSGYKFPLYMIGHGMLDSDLHLSSKAQVFEHPHIQDAASQLPDDESLFFGDTGLSKNPIELVEGWFSSWKSSIASFFFIIGLIIGLFLVLRVGIHLCIKLKHTKKRQIYTDIEMNRLGK

SEQ ID NO: 17 - protein, 494 aa, synthetic construct
KFSIVFPQSQKGNWKNVPSSYHYCPSSSDQNWHNDLLGITMKVKMPTHTAIQADGWMCHAAKWITTCDFRWYGPKYITHSIHSIQPTSEQCKESIKQTKQGTWMSPGFPPQNCGYATVTDSVAVVVQATPHHVLVDEYTGEWIDTQFPNGKCETEECETVHNSTVWYSDYKVTGLCDATLVDTEITFFSEDGKKESIGKPNTGYRSNYFAYENGDKVCKMNYCKHAGVRLPSGVWFEFVDQDVYAAAKLPECPVGATISAPTQTSVDVSLILDVERILDYSLCQETWSKIRSKQPVSPVDLSYLAPKNPGTGPAFTIINGTLKYFETRYIRIDIDNPIISKMVGKISGSQAERELWTEWFPYEGVEIGPNGILKTPTGYKFPLFMIGHGMLDSDLHKTSQAEVFEHPHLAEAPKQLPEEETLFFGDTGISKNPVELIEGWFSSWKSTVVTFFFAIGVFILLYVVARIVIAVRYRYQGSNNKRIYNDIEMSRFRK

SEQ ID NO: 18 - protein, 494 aa, synthetic construct
KFSIVFPQSQKGNWKNVPSSYHYCPSSSDQNWHNDLLGITMKVKMPTHKAIQADGWMCHAAKWITTCDFRWYGPKYITHSIHSIQPTSEQCKESIKQTKQGTWMSPGFPPQNCGYATVTDSVAVVVQATPHHVLVDEYTGEWIDSQFPNGKCETEECETVHNSTVWYSDYKVTGLCDATLVDTEITFFSEDGKKESIGKPNTGYRSNYFAYENGDKVCKMNYCKHAGVRLPSGVWFEFVDQDVYAAAKLPECPVGATISAPTQTSVDVSLILDVERILDYSLCQETWSKIRSKQPVSPVDLSYLAPKNPGTGPAFTIINGTLKYFETRYIRIDIDNPIISKMVGKISGSQAERELWTEWFPYEGVEIGPNGILKTPTGYKFPLFMIGHGMLDSDLHKTSQAEVFEHPHLAEAPKQLPEEETLFFGDTGISKNPVELIEGWFSSWKSTVVTFFFAIGVFILLYVVARIVIAVRYRYQGSNNKRIYNDIEMSRFRK

SEQ ID NO: 19 - protein, 495 aa, synthetic construct
KFSIVFPQSQKGNWKNVPSSYHYCPSSSDQNWHNDLLGITMKVKMPKTHTAIQADGWMCHAAKWITTCDFRWYGPKYITHSIHSIQPTSEQCKESIKQTKQGTWMSPGFPPQNCGYATVTDSVAVVVQATPHHVLVDEYTGEWIDTQFPNGKCETEECETVHNSTVWYSDYKVTGLCDATLVDTEITFFSEDGKKESIGKPNTGYRSNYFAYENGDKVCKMNYCKHAGVRLPSGVWFEFVDQDVYAAAKLPECPVGATISAPTQTSVDVSLILDVERILDYSLCQETWSKIRSKQPVSPVDLSYLAPKNPGTGPAFTIINGTLKYFETRYIRIDIDNPIISKMVGKISGSQAEQELWTEWFPYEGVEIGPNGILKTPTGYKFPLFMIGHGMLDSDLHKTSQAEVFEHPHLAEAPKQLPEEETLFFGDTGISKNPVELIEGWFSSWKSTVVTFFFAIGVFILLYVVARIVIAVRYRYQGSNNKRIYNDIEMSRFRK

SEQ ID NO: 20 - protein, 495 aa, synthetic construct
KFSIVFPQSQKGNWKNVPSSYHYCPSSSDQNWHNDLLGITMKVKMPKTHKAIQADGWMCHAAKWITTCDFRWYGPKYITHSIHSIQPTSEQCKESIKQTKQGTWMSPGFPPQNCGYATVTDSVAVVVQATPHHVLVDEYTGEWIDSQFPNGKCETEECETVHNSTVWYSDYKVTGLCDATLVDTEITFFSEDGKKESIGKPNTGYRSNYFAYENGDKVCKMNYCKHAGVRLPSGVWFEFVDQDVYAAAKLPECPVGATISAPTQTSVDVSLILDVERILDYSLCQETWSKIRSKQPVSPVDLSYLAPKNPGTGPAFTIINGTLKYFETRYIRIDIDNPIISKMVGKISGSQAEQELWTEWFPYEGVEIGPNGILKTPTGYKFPLFMIGHGMLDSDLHKTSQAEVFEHPHLAEAPKQLPEEETLFFGDTGISKNPVELIEGWFSSWKSTVVTFFFAIGVFILLYVVARIVIAVRYRYQGSNNKRIYNDIEMSRFRK

SEQ ID NO: 21 - protein, 126 aa, synthetic construct
DVQLQESGGGLVQAGGSLRLSCAASGRAFSVYAMAWFRQAPGKEREFVSSIAGSSSTYYTNYADSVKGRFTISRDNAKNTMYLQMDELKDEDTAVYYCAASPRSNNGRETRHYDYWGQGTQVTVSS

SEQ ID NO: 22 - protein, 10 aa, synthetic construct
GRAFSVYAMA

SEQ ID NO: 23 - protein, 12 aa, synthetic construct
SIAGSSSTYYTN

SEQ ID NO: 24 - protein, 15 aa, synthetic construct
SPRSNNGRETRHYDY

SEQ ID NO: 25 - protein, 511 aa, Vesicular Stomatitis Virus-Indiana
MKCLLYLAFLFIGVNCKFTIVFPHNQKGNWKNVPSNYHYCPSSSDLNWHNDLIGTALQVKMPKSHKAIQADGWMCHASKWVTTCDFRWYGPKYITHSIRSFTPSVEQCKESIEQTKQGTWLNPGFPPQSCGYATVTDAEAVIVQVTPHHVLVDEYTGEWVDSQFINGKCSNYICPTVHNSTTWHSDYKVKGLCDSNLISMDITFFSEDGELSSLGKEGTGFRSNYFAYETGGKACKMQYCKHWGVRLPSGVWFEMADKDLFAAARFPECPEGSSISAPSQTSVDVSLIQDVERILDYSLCQETWSKIRAGLPISPVDLSYLAPKNPGTGPAFTIINGTLKYFETRYIRVDIAAPILSRMVGMISGTTTERELWDDWAPYEDVEIGPNGVLRTSSGYKFPLYMIGHGMLDSDLHLSSKAQVFEHPHIQDAASQLPDDESLFFGDTGLSKNPIELVEGWFSSWKSSIASFFFIIGLIIGLFLVLRVGIHLCIKLKHTKKRQIYTDIEMNRLGK

SEQ ID NO: 26 - protein, 495 aa, synthetic construct
KFTIVFPHNQKGNWKNVPSNYHYCPSSSDLNWHNDLIGTALQVKMPKSHKAIQADGWMCHASKWVTTCDFRWYGPKYITHSIRSFTPSVEQCKESIEQTKQGTWLNPGFPPQSCGYATVTDAEAVIVQVTPHHVLVDEYTGEWVDSQFINGKCSNYICPTVHNSTTWHSDYKVKGLCDSNLISMDITFFSEDGELSSLGKEGTGFRSNYFAYETGGKACKMQYCKHWGVRLPSGVWFEMADKDLFAAARFPECPEGSSISAPSQTSVDVSLIQDVERILDYSLCQETWSKIRAGLPISPVDLSYLAPKNPGTGPAFTIINGTLKYFETRYIRVDIAAPILSRMVGMISGTTTEQELWDDWAPYEDVEIGPNGVLRTSSGYKFPLYMIGHGMLDSDLHLSSKAQVFEHPHIQDAASQLPDDESLFFGDTGLSKNPIELVEGWFSSWKSSIASFFFIIGLIIGLFLVLRVGIHLCIKLKHTKKRQIYTDIEMNRLGK

SEQ ID NO: 27 - protein, 512 aa, Vesicular Stomatitis Virus-Cocal
MNFLLLTFIVLPLCSHAKFSIVFPQSQKGNWKNVPSSYHYCPSSSDQNWHNDLLGITMKVKMPKTHKAIQADGWMCHAAKWITTCDFRWYGPKYITHSIHSIQPTSEQCKESIKQTKQGTWMSPGFPPQNCGYATVTDSVAVVVQATPHHVLVDEYTGEWIDSQFPNGKCETEECETVHNSTVWYSDYKVTGLCDATLVDTEITFFSEDGKKESIGKPNTGYRSNYFAYEKGDKVCKMNYCKHAGVRLPSGVWFEFVDQDVYAAAKLPECPVGATISAPTQTSVDVSLILDVERILDYSLCQETWSKIRSKQPVSPVDLSYLAPKNPGTGPAFTIINGTLKYFETRYIRIDIDNPIISKMVGKISGSQTERELWTEWFPYEGVEIGPNGILKTPTGYKFPLFMIGHGMLDSDLHKTSQAEVFEHPHLAEAPKQLPEEETLFFGDTGISKNPVELIEGWFSSWKSTVVTFFFAIGVFILLYVVARIVIAVRYRYQGSNNKRIYNDIEMSRFRK

SEQ ID NO: 28 - protein, 495 aa, synthetic construct
KFSIVFPQSQKGNWKNVPSSYHYCPSSSDQNWHNDLLGITMKVKMPKTHKAIQADGWMCHAAKWITTCDFRWYGPKYITHSIHSIQPTSEQCKESIKQTKQGTWMSPGFPPQNCGYATVTDSVAVVVQATPHHVLVDEYTGEWIDSQFPNGKCETEECETVHNSTVWYSDYKVTGLCDATLVDTEITFFSEDGKKESIGKPNTGYRSNYFAYEKGDKVCKMNYCKHAGVRLPSGVWFEFVDQDVYAAAKLPECPVGATISAPTQTSVDVSLILDVERILDYSLCQETWSKIRSKQPVSPVDLSYLAPKNPGTGPAFTIINGTLKYFETRYIRIDIDNPIISKMVGKISGSQTEQELWTEWFPYEGVEIGPNGILKTPTGYKFPLFMIGHGMLDSDLHKTSQAEVFEHPHLAEAPKQLPEEETLFFGDTGISKNPVELIEGWFSSWKSTVVTFFFAIGVFILLYVVARIVIAVRYRYQGSNNKRIYNDIEMSRFRK

SEQ ID NO: 29 - protein, 495 aa, synthetic construct
KFTIVFPHNQKGNWKNVPSNYHYCPSSSDLNWHNDLIGTALQVKMPKSHKAIQADGWMCHASKWVTTCDFRWYGPKYITHSIRSFTPSVEQCKESIEQTKQGTWLNPGFPPQSCGYATVTDAEAVIVQVTPHHVLVDEYTGEWVDSQFINGKCSNYICPTVHNSTTWHSDYKVKGLCDSNLISMDITFFSEDGELSSLGKEGTGFRSNYFAYENGGKACKMQYCKHWGVRLPSGVWFEMADKDLFAAARFPECPEGSSISAPSQTSVDVSLIQDVERILDYSLCQETWSKIRAGLPISPVDLSYLAPKNPGTGPAFTIINGTLKYFETRYIRVDIAAPILSRMVGMISGTTAERELWDDWAPYEDVEIGPNGVLRTSSGYKFPLYMIGHGMLDSDLHLSSKAQVFEHPHIQDAASQLPDDESLFFGDTGLSKNPIELVEGWFSSWKSSIASFFFIIGLIIGLFLVLRVGIHLCIKLKHTKKRQIYTDIEMNRLGK

SEQ ID NO: 30 - protein, 494 aa, synthetic construct
KFTIVFPHNQKGNWKNVPSNYHYCPSSSDLNWHNDLIGTALQVKMPSHKAIQADGWMCHASKWVTTCDFRWYGPKYITHSIRSFTPSVEQCKESIEQTKQGTWLNPGFPPQSCGYATVTDAEAVIVQVTPHHVLVDEYTGEWVDSQFINGKCSNYICPTVHNSTTWHSDYKVKGLCDSNLISMDITFFSEDGELSSLGKEGTGFRSNYFAYETGGKACKMQYCKHWGVRLPSGVWFEMADKDLFAAARFPECPEGSSISAPSQTSVDVSLIQDVERILDYSLCQETWSKIRAGLPISPVDLSYLAPKNPGTGPAFTIINGTLKYFETRYIRVDIAAPILSRMVGMISGTTTERELWDDWAPYEDVEIGPNGVLRTSSGYKFPLYMIGHGMLDSDLHLSSKAQVFEHPHIQDAASQLPDDESLFFGDTGLSKNPIELVEGWFSSWKSSIASFFFIIGLIIGLFLVLRVGIHLCIKLKHTKKRQIYTDIEMNRLGK